European Patent Specification EP 2 964 257 B1, published October 9, 2024. Title: TRANSCUTANEOUS DOSAGE FORMULATION. Applicant: BAKALETZ. The sequence listing filed with the application follows.

SEQUENCE LISTING (57 sequences)

SEQ ID NO: 1 - DNA, 4345 bp, H. influenzae
  CDS (403)..(849)
gcgatcattaaaattgacatattgcgtaattcgcccatttcgttcgatcaaacaatgtgctgaaacacgcatttgataaatttctgcaaaataaggatgaatcttaggatctaattttccttgaaaaaaatcatccacatatccgccgccaaattgttctggcggcagactaatataatgaataaccaataaggaaatatcctgtggatttgggcgtttatcgaagtgaggtgactgaatttgccgacaatccaatataccttgttcaatatcttttagtttttgcatacttttttcctttttttgcgatcaggatcgcagaaaaagtgcggtcaattttacaaacaaatttttccttttcacaatgtcgtcgctaacaaaggcttaataaaaggaaaatgaatgaaactaacaacacagcaaaccttgaaaaaagggtttacattaatagagctaatgattgtgattgcaattattgctattttagccactatcgcaattccctcttatcaaaattatactaaaaaagcagcggtatctgaattactgcaagcgtcagcgccttataaggctgatgtggaattatgtgtatatagcacaaatgaaacaacaaactgtacgggtggaaaaaatggtattgcagcagatataaccacagcaaaaggctatgtaaaatcagtgacaacaagcaacggtgcaataacagtaaaaggggatggcacattggcaaatatggaatatattttgcaagctacaggtaatgctgcaacaggtgtaacttggacaacaacttgcaaaggaacggatgcctctttatttccagcaaatttttgcggaagtgtcacacaatgacgagctatgctttacttcatactcagcgtgtaaccgctcaaaatggcgagatctttacgatctcgccagatttatgggaacgcaatcagcagcaacaatccttgctcttgcggtattttgctttgccacttaaagaagaaaataatcgtctttggctaggggttgattctctctccaatctttcagcttgtgaaaccattgcgtttataacaggaaaacctgtcgaaccaattttgttagaaagcagccaactcaaagaactgttacaacaacttactccgcaccaaatgcaagtggaagagcaagttaaattctatcaacatcaagaaacccattttgaacaagaagatgatgaacctgttatccgcttacttaatcagatttttgaatctgccttacaaaaaaatgcctctgatattcatttagaaaccttggctgatcagtttcaagtgcggtttagaattgatggtgttttacaaccacaacccttaataagcaaaatattcgccaatcgtattatttcacgcttaaaattactggctaaattagatattagtgaaaatcgacttccacaagatggacgatttcaatttaaaaccactttttccgatattcttgattttcgcctttcaaccttaccaacccattggggcgaaaaaatcgtgttgcgagcgcaacaaaataaacctgtagaacttagctttgctgaactgggtatgaccgaaaatcagcaacaagcatttcaacgctcacttagccagccacaaggattaattttagtaaccggccccacaggaagtgggaaaagtatctcgctttacaccgcacttcagtggctaaatacgcctgataaacatattatgaccgctgaagatcccattgaaattgaacttgatggtattattcaaagccaaattaatccgcagattggattagattttagccgtctattgcgtgcttttttacgtcaagatcccgacatcattatgctaggtgaaattcgagatgaagaaagtgcaaggattgcactacgtgccgctcaaacgggacatttggtgctttcaactttacataccaatgatgcaatatctgccatttctcgcttacaacaactcggtattcaacaacatgaaattgaaaacagtttactactcgtcattgcacagcgtcttgtacgaaaaatctgtccaaagtgcggtggaaatttaataaattcttgtgattgccatcaaggttatcgagggcgaatcggcgtgtatcaatttctacattggcaacagaatggctatcaaacggattttgagaatttacgagagagtggtttggaaaaagttagccaaggcataacagatgagaaagaaattgaacgtgtgttaggtaaaaactcatgactaaaaaactcttttattatcaaggtagtaacgcattaaatcagaaacaaaaaggctcaattattgcggatacgaaacaacaagcgcactttcagttaataagccgcgggcttactcacatcaaattacaacaaaactggcaatttggggcaaaacccaaaaattcagaaatcagtgaattactcaatcaattagcgacattgctacagtccgtaattccgttaaaaaacagcctacaaattttgcaacaaaattgtactcaaattatgctcaacaaatggcttgaacgactgcttcaatccattgaatctggcttagcattctcacaagccattgaacaacaaggaaaatatctcacacaacaagaaattcaactgattcaagtgggagaaatgacaggaaaacttgccgtagtttgtaaaaaaatagccacgcaccgtagtcaatctttggctttacaacgcaaattacagaaaattatgttatatccctcaatggtattgggaatttctctattattgacactcgcattactgctttttatcgcgcctcaatttgctgaaatgtacagtggcaataatgcggagttaccaacaataaccgcaatattgctctcaatatctaatttccttaagcaaaatattggcattttgctatttttcgttttgagtttttttctattttattatttctatctaaaacgccagacttggtttcatcaaaagaaaaatcaacttatttctatcacgcctatttttggcacaattcaaaagctttcacgtttagtgaactttagtcaaagtttacaaattatgttgcaggccggcgtaccgcttaatcaggcactagacagttttcttcctcgcacacaaacttggcaaaccaagaaaacgcttgtaaacgatatggtattagataaagaagtgcggtcaattttgcaatgggtttctcaaggctatgcgttttctaatagcgtaagtagcgatcttttcccgatggaagcacaacaaatgctacaaattggcgaacaaagcggaaaactcgctttgatgctagagcatatcgcagataattaccaagaaaaacttaatcatcaaattgacttactctcacaaatgctagaaccattaatgatggtaatcatcggcagtctgattgggattattatgatgggaatgtatttacctatctttaatatgggatcagttattcaatgatttacttcacaatgtttttattaggcggcatcttagggatcgcattgtggttctacctatctggttttattacgcatttgcagcaagagatttatgcgacttacgttgaattatttccacaaaacagttctccatttcaaccgcactttgcctctattcaacaaaaaaagtgcggtcatattttgaggtatttttttagtattggggttggatttatatttttacaaattgccttcaaagattctatttttactgtatggatcggactcacacttattattctttggacaatcagttatcttgattggcactatcaacttatttctacgacaccctgtttatggttacttactctcggtttatttggcgcagacaataacttttcattgctaacgttatctgaaagcataaaaagtgcggctagtttttttattgttttctacgcaatctattggattgcaaaatgttattatagaaaagaagcctttggacggggagattattggctagcaatggcattaggaagttttattcatttagaaaccttaccgcactttttattattagcctcagtgcttggaatatgtttttcgcttattcataaaaagaaaaaagaatttataccttttgccccttttatgaacttatcggctatcattatttatctcgtcaaatattacggatattaaaaaggggaaaacataatatttttcccttgttcttcatagaagtgcggttgtttttacgaacgtttcatcacttcaaaaaactcttcgttggttttcgccatcatcagcttatcaatcaagaattccattgcatccacttcatccattggattaagaatcttacgaagaatccacattttttgtaattcgtccgctg

SEQ ID NO: 2 - protein, 149 aa, H. influenzae
MKLTTQQTLKKGFTLIELMIVIAIIAILATIAIPSYQNYTKKAAVSELLQASAPYKADVELCVYSTNETTNCTGGKNGIAADITTAKGYVKSVTTSNGAITVKGDGTLANMEYILQATGNAATGVTWTTTCKGTDASLFPANFCGSVTQ

SEQ ID NO: 3 - protein, 131 aa, H. influenzae
MGSSHHHHHHSSGLVPRGSHMTKKAAVSELLQASAPYKADVELCVYSTNETTNCTGGKNGIAADITTAKGYVKSVTTSNGAITVKGDGTLANMEYILQATGNAATGVTWTTTCKGTDASLFPANFCGSVTQ

SEQ ID NO: 4 - protein, 19 aa, Artificial sequence
  Synthetic Peptide
RSDYKFYEDANGTRDHKKG

SEQ ID NO: 5 - protein, 24 aa, Artificial sequence
  Synthetic Peptide
LVRSDYKFYEDANGTRDHKKGRHT

SEQ ID NO: 6 - protein, 22 aa, Artificial Sequence
  Synthetic Peptide
RSDYKLYNKNSSSNSTLKNLGE

SEQ ID NO: 7 - protein, 19 aa, Artificial sequence
  Synthetic Peptide
RSDYKLYNKNSSTLKDLGE

SEQ ID NO: 8 - protein, 13 aa, Artificial sequence
  Synthetic Peptide
RSDYKFYDNKRID

SEQ ID NO: 9 - protein, 139 aa, Artificial sequence
  Chimeric protein
MGSSHHHHHSSGLVPRGSHMTKKAAVSELLQASAPYKADVELCRSDYKFYEDANGTRDHKKGCTGGKNGIAADITTAKGYVKSVTTSNGAITVKGDGTLANMEYILQATGNAATGVTWTTCKGTDASLFPANFCGSVTQ

SEQ ID NO: 10 - protein, 143 aa, Artificial sequence
  Chimeric Protein
MGSSHHHHHSSGLVPRGSHMTKKAAVSELLQASAPYKADVELCLVRSDYKFYEDANGTRDHKKGHTCTGGKNGIAADITTAKGYVKSVTTSNGAITVKGDGTLANMEYILQATGNAATGVTWTTCKGTDASLFPANFCGSVTQ

SEQ ID NO: 11 - protein, 136 aa, Artificial sequence
  Chimeric Protein
MGSSHHHHHSSGLVPRGSHMTKKAAVSELLQASAPYKADVELCVTSTNETTNCTGGKNGIAADITTAKGYVKSVTTSNGAITVKGDGTLANMEYILQATGNAATGVTWTTCRSDYKFYEDANGTRDHKKGCGSVTQ

SEQ ID NO: 12 - protein, 141 aa, Artificial sequence
  Chimeric Protein
MGSSHHHHHSSGLVPRGSHMTKKAAVSELLQASAPYKADVELCVTSTNETTNCTGGKNGIAADITTAKGYVKSVTTSNGAITVKGDGTLANMEYILQATGNAATGVTWTTCLVRSDYKFYEDANGTRDHKKGRHTCGSVTQ

SEQ ID NO: 13 - protein, 148 aa, Artificial sequence
  Chimeric Protein
MGSSHHHHHSSGLVPRGSHMTKKAAVSELLQASAPYKADVELCVTSTNETTNCTGGKNGIAADITTAKGYVKSVTTSNGAITVKGDGTLANMEYILQATGNAATGVTWTTCKGTDASLFPANFCGSVTQRSDYKFYEDANGTRDHKKG

SEQ ID NO: 14 - protein, 153 aa, Artificial sequence
  Chimeric Protein
MGSSHHHHHSSGLVPRGSHMTKKAAVSELLQASAPYKADVELCVTSTNETTNCTGGKNGIAADITTAKGYVKSVTTSNGAITVKGDGTLANMEYILQATGNAATGVTWTTCKGTDASLFPANFCGSVTQLVRSDYKFYEDANGTRDHKKGRHT

SEQ ID NO: 15 - protein, 142 aa, Artificial sequence
  Chimeric Protein
MGSSHHHHHSSGLVPRGSHMTKKAAVSELLQASAPYKADVELCRSDYKLYNKNSSSNSTLKNLGECTGGKNGIAADITTAKGYVKSVTTSNGAITVKGDGTLANMEYILQATGNAATGVTWTTCKGTDASLFPANFCGSVTQ

SEQ ID NO: 16 - protein, 147 aa, Artificial sequence
  Chimeric Protein
MGSSHHHHHSSGLVPRGSHMTKKAAVSELLQASAPYKADVELCLVRSDYKLYNKNSSSNSTLKNLGERHTCTGGKNGIAADITTAKGYVKSVTTSNGAITVKGDGTLANMEYILQATGNAATGVTWTTCKGTDASLFPANFCGSVTQ

SEQ ID NO: 17 - protein, 139 aa, Artificial sequence
  Chimeric Protein
MGSSHHHHHSSGLVPRGSHMTKKAAVSELLQASAPYKADVELCVTSTNETTNCTGGKNGIAADITTAKGYVKSVTTSNGAITVKGDGTLANMEYILQATGNAATGVTWTTCRSDYKLYNKNSSSNSTLKNLGECGSVTQ

SEQ ID NO: 18 - protein, 144 aa, Artificial sequence
  Chimeric Protein
MGSSHHHHHSSGLVPRGSHMTKKAAVSELLQASAPYKADVELCVTSTNETTNCTGGKNGIAADITTAKGYVKSVTTSNGAITVKGDGTLANMEYILQATGNAATGVTWTTCLVRSDYKLYNKNSSSNSTLKNLGERHTCGSVTQ

SEQ ID NO: 19 - protein, 151 aa, Artificial sequence
  Chimeric Protein
MGSSHHHHHSSGLVPRGSHMTKKAAVSELLQASAPYKADVELCVTSTNETTNCTGGKNGIAADITTAKGYVKSVTTSNGAITVKGDGTLANMEYILQATGNAATGVTWTTCKGTDASLFPANFCGSVTQRSDYKLYNKNSSSNSTLKNLGE

SEQ ID NO: 20 - protein, 156 aa, Artificial sequence
  Chimeric Protein
MGSSHHHHHSSGLVPRGSHMTKKAAVSELLQASAPYKADVELCVTSTNETTNCTGGKNGIAADITTAKGYVKSVTTSNGAITVKGDGTLANMEYILQATGNAATGVTWTTCKGTDASLFPANFCGSVTQLVRSDYKLYNKNSSSNSTLKNLGERHT

SEQ ID NO: 21 - protein, 139 aa, Artificial sequence
  Chimeric Protein
MGSSHHHHHSSGLVPRGSHMTKKAAVSELLQASAPYKADVELCRSDYKLYNKNSSSLKNLGECTGGKNGIAADITTAKGYVKSVTTSNGAITVKGDGTLANMEYILQATGNAATGVTWTTCKGTDASLFPANFCGSVTQ

SEQ ID NO: 22 - protein, 145 aa, Artificial sequence
  Chimeric Protein
MGSSHHHHHSSGLVPRGSHMTKKAAVSELLQASAPYKADVELCLVRSDYKLYNKNSSSTLKNLGERHTCTGGKNGIAADITTAKGYVKSVTTSNGAITVKGDGTLANMEYILQATGNAATGVTWTTCKGTDASLFPANFCGSVTQ

SEQ ID NO: 23 - protein, 136 aa, Artificial sequence
  Chimeric Protein
MGSSHHHHHSSGLVPRGSHMTKKAAVSELLQASAPYKADVELCVTSTNETTNCTGGKNGIAADITTAKGYVKSVTTSNGAITVKGDGTLANMEYILQATGNAATGVTWTTCRSDYKLYNKNSSTLKNLGECGSVTQ

SEQ ID NO: 24 - protein, 141 aa, Artificial sequence
  Chimeric Protein
MGSSHHHHHSSGLVPRGSHMTKKAAVSELLQASAPYKADVELCVTSTNETTNCTGGKNGIAADITTAKGYVKSVTTSNGAITVKGDGTLANMEYILQATGNAATGVTWTTCLVRSDYKLYNKNSSTLKNLGERHTCGSVTQ

SEQ ID NO: 25 - protein, 148 aa, Artificial sequence
  Chimeric Protein
MGSSHHHHHSSGLVPRGSHMTKKAAVSELLQASAPYKADVELCVTSTNETTNCTGGKNGIAADITTAKGYVKSVTTSNGAITVKGDGTLANMEYILQATGNAATGVTWTTCKGTDASLFPANFCGSVTQRSDYKLYNKNSSTLKNLGE

SEQ ID NO: 26 - protein, 153 aa, Artificial sequence
  Chimeric Protein
MGSSHHHHHSSGLVPRGSHMTKKAAVSELLQASAPYKADVELCVTSTNETTNCTGGKNGIAADITTAKGYVKSVTTSNGAITVKGDGTLANMEYILQATGNAATGVTWTTCKGTDASLFPANFCGSVTQLVRSDYKLYNKNSSTLKNLGERHT

SEQ ID NO: 27 - protein, 133 aa, Artificial sequence
  Chimeric Protein
MGSSHHHHHSSGLVPRGSHMTKKAAVSELLQASAPYKADVELCRSDYKFYDNKRIDCTGGKNGIAADITTAKGYVKSVTTSNGAITVKGDGTLANMEYILQATGNAATGVTWTTCKGTDASLFPANFCGSVTQ

SEQ ID NO: 28 - protein, 138 aa, Artificial sequence
  Chimeric Protein
MGSSHHHHHSSGLVPRGSHMTKKAAVSELLQASAPYKADVELCLVRSDYKFYDNKRIDRHTCTGGKNGIAADITTAKGYVKSVTTSNGAITVKGDGTLANMEYILQATGNAATGVTWTTCKGTDASLFPANFCGSVTQ

SEQ ID NO: 29 - protein, 130 aa, Artificial sequence
  Chimeric Protein
MGSSHHHHHSSGLVPRGSHMTKKAAVSELLQASAPYKADVELCVTSTNETTNCTGGKNGIAADITTAKGYVKSVTTSNGAITVKGDGTLANMEYILQATGNAATGVTWTTCRSDYKFYDNKRIDCGSVTQ

SEQ ID NO: 30 - protein, 135 aa, Artificial sequence
  Chimeric Protein
MGSSHHHHHSSGLVPRGSHMTKKAAVSELLQASAPYKADVELCVTSTNETTNCTGGKNGIAADITTAKGYVKSVTTSNGAITVKGDGTLANMEYILQATGNAATGVTWTTCLVRSDYKFYDNKRIDRHTCGSVTQ

SEQ ID NO: 31 - protein, 142 aa, Artificial sequence
  Chimeric Protein
MGSSHHHHHSSGLVPRGSHMTKKAAVSELLQASAPYKADVELCVTSTNETTNCTGGKNGIAADITTAKGYVKSVTTSNGAITVKGDGTLANMEYILQATGNAATGVTWTTCKGTDASLFPANFCGSVTQRSDYKFYDNKRID

SEQ ID NO: 32 - protein, 147 aa, Artificial sequence
  Chimeric Protein
MGSSHHHHHSSGLVPRGSHMTKKAAVSELLQASAPYKADVELCVTSTNETTNCTGGKNGIAADITTAKGYVKSVTTSNGAITVKGDGTLANMEYILQATGNAATGVTWTTCKGTDASLFPANFCGSVTQLVRSDYKFYDNKRIDRHT

SEQ ID NO: 33 - DNA, 447 bp, H. influenzae
  CDS (1)..(447)
atgaaattaacaacacagcaaaccttgaaaaaagggtttacattaatagagctaatgattgtgattgcaattattgctattttagccactatcgcaattccctcttatcaaaattatactaaaaaagcagcggtatctgaattactgcaagcgtcagcgccttataaggctgatgtggaattatgtgtatatagcacaaatgaaacaacaaactgtacgggtggaaaaaatggtattgcagcagatataaccacagcaaaaggctatgtaaaatcagtgacaacaagcaacggtgcaataacagtaaaaggggatggcacattggcaaatatggaatatattttgcaagctacaggtaatgctgcaacaggtgtaacttggacaacaacttgcaaaggaacggatgcctctttatttccagcaaatttttgcggaagtgtcacacaa

SEQ ID NO: 34 - protein, 149 aa, H. influenzae; identical to SEQ ID NO: 2

SEQ ID NO: 35 - DNA, 447 bp, H. influenzae; identical to SEQ ID NO: 33
  CDS (1)..(447)

SEQ ID NO: 36 - protein, 149 aa, H. influenzae; identical to SEQ ID NO: 2

SEQ ID NO: 37 - DNA, 447 bp, H. influenzae; identical to SEQ ID NO: 33
  CDS (1)..(447)

SEQ ID NO: 38 - protein, 149 aa, H. influenzae; identical to SEQ ID NO: 2

SEQ ID NO: 39 - DNA, 447 bp, H. influenzae; identical to SEQ ID NO: 33
  CDS (1)..(447)

SEQ ID NO: 40 - protein, 149 aa, H. influenzae; identical to SEQ ID NO: 2

SEQ ID NO: 41 - DNA, 447 bp, H. influenzae
  CDS (1)..(447)
atgaaattaacaacacagcaaaccttgaaaaaaggttttacattaatcgagctaatgattgtgattgcaattattgctattttagccactatcgcaattccttcttatcaaaattataccaaaaaagcttcggtatccgaattactgcaagcatctgcaccttataaggctgatgtggaattatgtgtatatagcacaaatgaaacaacaaactgtacgggtggaaaaaatggtattgcagctgatattacaacagcaaaaggctatgtagcctcagtgaaaactcaatcgggtggcattacagtaaaagggaatggcacattggcaaatatggaatatattttgcaagctaaaggtaatgctacagcaggtgtaacttggacaacaacctgcaaaggaacggatgcctctttatttccagcaaatttttgcagaagtgtcacaaaa

SEQ ID NO: 42 - protein, 149 aa, H. influenzae
MKLTTQQTLKKGFTLIELMIVIAIIAILATIAIPSYQNYTKKASVSELLQASAPYKADVELCVYSTNETTNCTGGKNGIAADITTAKGYVASVKTQSGGITVKGNGTLANMEYILQAKGNATAGVTWTTTCKGTDASLFPANFCRSVTK

SEQ ID NO: 43 - DNA, 447 bp, H. influenzae
  CDS (1)..(447)
atgaaattaacaacacagcaaaccttgaaaaaagggtttacattaatagagctaatgattgtgattgcaattattgctattttagccaccatcgcaattccttcttataaaaattatactaaaaaagcagcggtatctgaattactgcaagcttctgcgccttataaggctgatgtggaattatgtgtatatagcacaaatgaaataacaaattgtatgggtggaaaaaatggtattgcagctgatattacaacagcaaaaggctatgtagcctcagtgaaaactcaatcgggtggcattaccgtaaaaggggatggcacattggcaaatatggaatatattttgcaagctacaggtaatgctgcagcaggtgtaacttggacaacaacctgcaaaggaacggatgcctctttatttccagcaaatttttgcggaagtatcacacaa

SEQ ID NO: 44 - protein, 149 aa, H. influenzae
MKLTTQQTLKKGFTLIELMIVIAIIAILATIAIPSYKNYTKKAAVSELLQASAPYKADVELCVYSTNEITNCMGGKNGIAADITTAKGYVASVKTQSGGITVKGDGTLANMEYILQATGNAAAGVTWTTTCKGTDASLFPANFCGSITQ

SEQ ID NO: 45 - DNA, 447 bp, H. influenzae
  CDS (1)..(447)
atgaaattaacaacactgcaaaccttgaaaaaagggtttacattaatcgagctaatgattgtgattgcaattattgctattttagccactatcgcaattccttcttatcaaaattataccaaaaaagctgcggtatccgaattactgcaagcttctgcgccttataaggctgatgtggaattatgcgtttatagcacaggcaaaccttctacttgctcaggaggaagcaatggaattgcagctgatattacgacagcaaaaggctatgtagcctcagtgaaaactcaatcaggtggtattacagtaaaagggaatggcacattggcaaatatggaatatattttgcaagctacaggtaatgctgcaacaggtgtaacttggacaacaacttgcaaaggaacggatgcctctttatttccagcaaatttttgcggaagtgtcacacaa

SEQ ID NO: 46 - protein, 149 aa, H. influenzae
MKLTTLQTLKKGFTLIELMIVIAIIAILATIAIPSYQNYTKKAAVSELLQASAPYKADVELCVYSTGKPSTCSGGSNGIAADITTAKGYVASVKTQSGGITVKGNGTLANMEYILQATGNAATGVTWTTTCKGTDASLFPANFCGSVTQ

SEQ ID NO: 47 - DNA, 447 bp, H. influenzae
  CDS (1)..(447)
atgaaattaacaacactgcaaaccttgaaaaaagggtttacattaatcgagctaatgattgtgattgcaattattgctattttagccactatcgcaattccttcttatcaaaattataccaaaaaagctgcggtatccgaattactgcaagcttctgcgccttataaggctgatgtggaattatgcgtttatagcacaggcaaactttctacttgctcaggaggaagcaatggaattgcagctgatattacaacagcaaaaggctatgtagcctcagtgaaaactcaatcaggtggtattacagtaaaagggaatggcacattggcaaatatggaatatattttgcaagctaaaggtaatgctacagcaggtgtaacttggacaacaacctgcaaaggaacggatgcctctttatttccagcaaatttttgcggaagtgtcacaaaa

SEQ ID NO: 48 - protein, 149 aa, H. influenzae
MKLTTLQTLKKGFTLIELMIVIAIIAILATIAIPSYQNYTKKAAVSELLQASAPYKADVELCVYSTGKLSTCSGGSNGIAADITTAKGYVASVKTQSGGITVKGNGTLANMEYILQAKGNATAGVTWTTTCKGTDASLFPANFCGSVTK

SEQ ID NO: 49 - DNA, 447 bp, H. influenzae
  CDS (1)..(447)
atgaaattaacaacacagcaaaccttgaaaaaaggttttacattaatcgagctaatgattgtgattgcaattattgctattttagccactatcgcaattccttcttatcaaaattataccaaaaaagcttcggtatccgaattactgcaagcttccgcaccttataagtcagatgtggaattatgcgtttatagcacaggcaaaccttctacttgctcaggaggaagcaatggaattgcagctgatattacaacagcaaaaggctatgtagcctcagtgaaaactcaatcaggtggtattacagtaaaagggaatggcacattggcaaatatggaatatattttgcaagctaaaggtaatgctacagcaggtgtaacttggacaacaacctgcaaaggaacggatgcctctttatttccagcaaatttttgcagaagtgtcacaaaa

SEQ ID NO: 50 - protein, 149 aa, H. influenzae
MKLTTQQTLKKGFTLIELMIVIAIIAILATIAIPSYQNYTKKASVSELLQASAPYKSDVELCVYSTGKPSTCSGGSNGIAADITTAKGYVASVKTQSGGITVKGNGTLANMEYILQAKGNATAGVTWTTTCKGTDASLFPANFCRSVTK

SEQ ID NO: 51 - DNA, 447 bp, H. influenzae
  CDS (1)..(447)
atgaaattaacaacacagcaaaccttgaaaaaagggtttacattaatagagctaatgattgtgattgcaattattgctattttagccactatcgcaattccctcttatcaaaattatactaaaaaagcggcggtatctgaattactgcaagcgtcagcgccttataaggctgatgtggaattatgtgtatatagtacaggtaaaccttccagttgctcgggaggaagcaatggaattgcggctgatattacaacagcaaaaggctatgtaaaatcagtgacaacaagcaacggtgcaataacagtaaaaggggatggcacattggcaaatatggaatatattttgcaagccagtggtaatgctgcaacaggtgtaacttggacaacaacttgcaaaggaacggatgcctctttatttccagcaaatttttgcggaagtgtcacacaa

SEQ ID NO: 52 - protein, 149 aa, H. influenzae
MKLTTQQTLKKGFTLIELMIVIAIIAILATIAIPSYQNYTKKAAVSELLQASAPYKADVELCVYSTGKPSSCSGGSNGIAADITTAKGYVKSVTTSNGAITVKGDGTLANMEYILQASGNAATGVTWTTTCKGTDASLFPANFCGSVTQ

SEQ ID NO: 53 - protein, 40 aa, Artificial sequence
  Synthetic Peptide
RSDYKFYEDANGTRDHKKGPSLKLLSLIKGVIVHRLEGVE

SEQ ID NO: 54 - protein, 129 aa, Artificial sequence
  Chimeric protein
GSHMTKKAAVSELLQASAPYKADVELCLVRSDYKFYEDANGTRDHKKGRHTCTGGKNGIAADITTAKGYVKSVTTSNGAITVKGDGTLANMEYILQATGNAATGVTWTTTCKGTDASLFPANFCGSVTQ

SEQ ID NO: 55 - protein, 126 aa, Artificial sequence
  Chimeric protein
GSHMTKKAAVSELLQASAPYKADVELCVYSTNETTNCTGGKNGIAADITTAKGYVKSVTTSNGAITVKGDGTLANMEYILQATGNAATGVTWTTTCLVRSDYKFYEDANGTRDHKKGRHTCGSVTQ

SEQ ID NO: 56 - protein, 138 aa, Artificial sequence
  Chimeric protein
GSHMTKKAAVSELLQASAPYKADVELCVYSTNETTNCTGGKNGIAADITTAKGYVKSVTTSNGAITVKGDGTLANMEYILQATGNAATGVTWTTTCKGTDASLFPANFCGSVTQLVRSDYKFYEDANGTRDHKKGRHT

SEQ ID NO: 57 - protein, 144 aa, Artificial sequence
  Chimeric protein
GSHMLVRSDYKFYEDANGTRDHKKGRHTGPSLKLTKKAAVSELLQASAPYKADVELCVYSTNETTNCTGGKNGIAADITTAKGYVKSVTTSNGAITVKGDGTLANMEYILQATGNAATGVTWTTTCKGTDASLFPANFCGSVTQ